European Patent Specification EP 3 630 748 B1, published April 19, 2023. Title: IRE1 SMALL MOLECULE INHIBITORS. Applicant: QUENTIS THERAPEUTICS, INC. The sequence listing filed with the application follows.

SEQUENCE LISTING (7 sequences)

SEQ ID NO: 1 - protein, 977 aa, Homo sapiens
MPARRLLLLLTLLLPGLGIFGSTSTVTLPETLLFVSTLDGSLHAVSKRTGSIKWTLKEDPVLQVPTHVEEPAFLPDPNDGSLYTLGSKNNEGLTKLPFTIPELVQASPCRSSDGILYMGKKQDIWYVIDLLTGEKQQTLSSAFADSLCPSTSLLYLGRTEYTITMYDTKTRELRWNATYFDYAASLPEDDVDYKMSHFVSNGDGLVVTVDSESGDVLWIQNYASPVVAFYVWQREGLRKVMHINVAVETLRYLTFMSGEVGRITKWKYPFPKETEAKSKLTPTLYVGKYSTSLYASPSMVHEGVAVVPRGSTLPLLEGPQTDGVTIGDKGECVITPSTDVKFDPGLKSKNKLNYLRNYWLLIGHHETPLSASTKMLERFPNNLPKHRENVIPADSEKKSFEEVINLVDQTSENAPTTVSRDVEEKPAHAPARPEAPVDSMLKDMATIILSTFLLIGWVAFIITYPLSMHQQQQLQHQQFQKELEKIQLLQQQQQQLPFHPPGDTAQDGELLDTSGPYSESSGTSSPSTSPRASNHSLCSGSSASKAGSSPSLEQDDGDEETSVVIVGKISFCPKDVLGHGAEGTIVYRGMFDNRDVAVKRILPECFSFADREVQLLRESDEHPNVIRYFCTEKDRQFQYIAIELCAATLQEYVEQKDFAHLGLEPITLLQQTTSGLAHLHSLNIVHRDLKPHNILISMPNAHGKIKAMISDFGLCKKLAVGRHSFSRRSGVPGTEGWIAPEMLSEDCKENPTYTVDIFSAGCVFYYVISEGSHPFGKSLQRQANILLGACSLDCLHPEKHEDVIARELIEKMIAMDPQKRPSAKHVLKHPFFWSLEKQLQFFQDVSDRIEKESLDGPIVKQLERGGRAVVKMDWRENITVPLQTDLRKFRTYKGGSVRDLLRAMRNKKHHYRELPAEVRETLGSLPDDFVCYFTSRFPHLLAHTYRAMELCSHERLFQPYYFHEPPEPQPPVTPDAL

SEQ ID NO: 2 - RNA, 17 nt, Artificial Sequence
  Description of Artificial Sequence: Synthetic probe
cauguccgcagcacaug

SEQ ID NO: 3 - RNA, 17 nt, Artificial Sequence
  Description of Artificial Sequence: Synthetic probe
cauguccccagcacaug

SEQ ID NO: 4 - protein, 434 aa, Saccharomyces cerevisiae
SRIANIPNFEQSLKNLVVSEKILGYGSSGTVVFQGSFQGRPVAVKRMLIDFCDIALMEIKLLTESDDHPNVIRYYCSETTDRFLYIALELCNLNLQDLVESKNVSDENLKLQKEYNPISLLRQIASGVAHLHSLKIIHRDLKPQNILVSTSSRFTADQQTGAENLRILISDFGLCKKLDSGQSSFRTNLNNPSGTSGWRAPELLEESNNLQTKRRLTRSIDIFSMGCVFYYILSKGKHPFGDKYSRESNIIRGIFSLDEMKCLHDRSLIAEATDLISQMIDHDPLKRPTAMKVLRHPLFWPKSKKLEFLLKVSDRLEIENRDPPSALLMKFDAGSDFVIPSGDWTVKFDKIFMDNLERYRKYHSSKLMDLLRALRNKYHHFMDLPEDIAELMGPVPDGFYDYFIKRFPNLLIGVYMIVKENLSDDQILREFLYS

SEQ ID NO: 5 - protein, 424 aa, Homo sapiens
DDGDEETSVVIVGKISFCPKDVLGHGAEGTIVYRGMFDNRDVAVKRILPECFSFADREVQLLRESDEHPNVIRYFCTEKDRQFQYIAIELCAATLQEYVEQKDCFAHLGLEPITLLQQTTSGLAHLHSLNIVHRDLKPHNILISMPNAHGKIKAMISDFGLCKKLAVGRHSFSRRSGVPGTEGWIAPEMLSEDCKENPTYTVDIFSAGCVFYYVVSEGSHPFGKSLQRQANILLGACSLDCLHPEKHEDVIARELIEKMIAMDPQKRPSANDVLKHPFFWSLEKQLQFFQDVSDRIEKESLDGPIVKQLERGGRAVVKMDWRENITDPLQTDLRKFRTYKGGSVRDLLRAMRNKKHHYRDLPEEVRETLGTLPDDFVCYFTSRFPHLLAHTYRAMELCSHERLFQPYYFHEPPEPQPPVTPDAL

SEQ ID NO: 6 - protein, 423 aa, Mus musculus
DDEDEETRMVIVGKISFCPKDVLGHGAEGTIVYKGMFDNRDVAVKRILPECFSFADREVQLLRESDEHPNVIRYFCTEKDRQFQYIAIELCAATLQEYVEQKDFAHLGLEPITLLHQTTSGLAHLHSLNIVHRDLKPHNILLSMPNAHGRIKAMISDFGLCKKLAVGRHSFSRRSGVPGTEGWIAPEMLSEDCKDNPTYTVDIFSAGCVFYYVISEGNHPFGKSLQRQANILLGACNLDCFHSDKHEDVIARELIEKMIAMDPQQRPSAKHVLKHPFFWSLEKQLQFFQDVSDRIEKEALDGPIVRQLERGGRAVVKMDWRENITVPLQTDLRKFRTYKGGSVRDLLRAMRNKKHHYRELPAEVQETLGSIPDDFVRYFTSRFPHLLSHTYQAMELCRHERLFQTYYWHEPTEPQPPVIPYAL

SEQ ID NO: 7 - protein, 423 aa, Rattus norvegicus
DDEDEETRMVIVGKISFCPKDVLGHGAEGTIVYKGMFDNRDVAVKRILPECFSFADREVQLLRESDEHPNVIRYFCTEKDRQFQYIAIELCAATLQEYVEQKDFAHLGLEPITLLHQTTSGLAHLHSLNIVHRDLKPHNILLSMPNAHGRIKAMISDFGLCKKLAVGRHSFSRRSGVPGTEGWIAPEMLSEDCKENPTYTVDIFSAGCVFYYVISEGNHPFGKSLQRQANILLGACSLDCFHSDKHEDVIARELIEKMIAMDPQQRPSAKHVLKHPFFWSLEKQLQFFQDVSDRIEKESLDGPIVRQLERGGRAVVKMDWRENITVPLQTDLRKFRTYKGGSVRDLLRAMRNKRHHYRELPLEVQETLGSIPDDFVRYFTSRFPHLLSHTYRAMELCRHERLFQTYYWHEPTEAQPPGIPDAL